European Patent Specification EP 3 525 813 B1, published April 17, 2024. Title: BROADLY NEUTRALIZING ANTIBODY TARGETING THE EBOLAVIRUS GLYCOPROTEIN INTERNAL FUSION LOOP. Applicant: Integrated BioTherapeutics, Inc. The University of Maryland AMAN, Mohammad Javad HOWELL, Katie A HOLTSBERG, Frederick Wayne ZHAO, Xuelian LI, Yuxing. The sequence listing filed with the application follows.

SEQUENCE LISTING (35 sequences)

SEQ ID NO: 1 - protein, 128 aa, cynomolgus macaque
QVQLQEWGEGLVKPSETLSLTCAVYGGSISGYYHWNWIRLPPGKGLEWIGNIDNSASTNYNPSLKTRVTISKDTSKNQISLKVRSLTAADTAVYYCARDPGFTIFGVVITSWSGLDSWGQGAVVTVSS

SEQ ID NO: 2 - protein, 106 aa, cynomolgus macaque
DIQMTQSPSSLSASVGDTVTITCRASQSISNNLAWYQQRPRRAPQLLIYAASNLASGVPSRFSGSGSGTDFTLTISSLQAEDFAAYYCQQHNTLPLTFGGGTKVEI

SEQ ID NO: 3 - protein, 6 aa, cynomolgus macaque
GYYHWN

SEQ ID NO: 4 - protein, 17 aa, cynomolgus macaque
GNIDNSASTNYNPSLKT

SEQ ID NO: 5 - protein, 19 aa, cynomolgus macaque
DPGFTIFGVVITSWSGLDS

SEQ ID NO: 6 - protein, 11 aa, cynomolgus macaque
RASQSISNNLA

SEQ ID NO: 7 - protein, 6 aa, cynomolgus macaque
AASNLA

SEQ ID NO: 8 - protein, 9 aa, cynomolgus macaque
QQHNTLPLT

SEQ ID NO: 9 - protein, 6 aa, cynomolgus macaque
  misc_feature (1)..(6): X is any amino acid
GYYXWX

SEQ ID NO: 10 - protein, 19 aa, cynomolgus macaque
  misc_feature (1)..(19): X is any amino acid
DXGXTIFXXXIXXWXXXDX

SEQ ID NO: 11 - protein, 676 aa, Ebola virus
MGVTGILQLPRDRFKRTSFFLWVIILFQRTFSIPLGVIHNSTLQVSDVDKLVCRDKLSSTNQLRSVGLNLEGNGVATDVPSVTKRWGFRSGVPPKVVNYEAGEWAENCYNLEIKKPDGSECLPAAPDGIRGFPRCRYVHKVSGTGPCAGDFAFHKEGAFFLYDRLASTVIYRGTTFAEGVVAFLILPQAKKDFFSSHPLREPVNATEDPSSGYYSTTIRYQATGFGTNETEYLFEVDNLTYVQLESRFTPQFLLQLNETIYASGKRSNTTGKLIWKVNPEIDTTIGEWAFWETKKNLTRKIRSEELSFTAVSNGPKNISGQSPARTSSDPETNTTNEDHKIMASENSSAMVQVHSQGRKAAVSHLTTLATISTSPQPPTTKTGPDNSTHNTPVYKLDISEATQVGQHHRRADNDSTASDTPPATTAAGPLKAENTNTSKSADSLDLATTTSPQNYSETAGNNNTHHQDTGEESASSGKLGLITNTIAGVAGLITGGRRTRREVIVNAQPKCNPNLHYWTTQDEGAAIGLAWIPYFGPAAEGIYTEGLMHNQDGLICGLRQLANETTQALQLFLRATTELRTFSILNRKAIDFLLQRWGGTCHILGPDCCIEPHDWTKNITDRIDQIIHDFVDKTLPDQGDNDNWWTGWRQWIPAGIGVTGVIIAVIALFCICKFVF

SEQ ID NO: 12 - protein, 676 aa, Ebola virus
MGVTGILQLPRDRFKRTSFFLWVIILFQRTFSIPLGVIHNSTLQVSDVDKLVCRDKLSSTNQLRSVGLNLEGNGVATDVPSATKRWGFRSGVPPKVVNYEAGEWAENCYNLEIKKPDGSECLPAAPDGIRGFPRCRYVHKVSGTGPCAGDFAFHKEGAFFLYDRLASTVIYRGTTFAEGVVAFLILPQAKKDFFSSHPLREPVNATEDPSSGYYSTTIRYQATGFGTNETEYLFEVDNLTYVQLESRFTPQFLLQLNETIYTSGKRSNTTGKLIWKVNPEIDTTIGEWAFWETKKNLTRKIRSEELSFTVVSNGAKNISGQSPARTSSDPGTNTTTEDHKIMASENSSAMVQVHSQGREAAVSHLTTLATISTSPQSLTTKPGPDNSTHNTPVYKLDISEATQVEQHHRRTDNDSTASDTPSATTAAGPPKAENTNTSKSTDFLDPATTTSPQNHSETAGNNNTHHQDTGEESASSGKLGLITNTIAGVAGLITGGRRTRREAIVNAQPKCNPNLHYWTTQDEGAAIGLAWIPYFGPAAEGIYIEGLMHNQDGLICGLRQLANETTQALQLFLRATTELRTFSILNRKAIDFLLQRWGGTCHILGPDCCIEPHDWTKNITDKIDQIIHDFVDKTLPDQGDNDNWWTGWRQWIPAGIGVTGVIIAVIALFCICKFVF

SEQ ID NO: 13 - protein, 676 aa, Ebola virus
MGVTGILQLPRDRFKRTSFFLWVIILFQRTFSIPLGVIHNSTLQVSDVDKLVCRDKLSSTNQLRSVGLNLEGNGVATDVPSATKRWGFRSGVPPKVVNYEAGEWAENCYNLEIKKPDGSECLPAAPDGIRGFPRCRYVHKVSGTGPCAGDFAFHKEGAFFLYDRLASTVIYRGTTFAEGVVAFLILPQAKKDFFSSHPLREPVNATEDPSSGYYSTTIRYQATGFGTNETEYLFEVDNLTYVQLESRFTPQFLLQLNETIYTSGKRSNTTGKLIWKVNPEIDTTIGEWAFWETKKNLTRKIRSEELSFTAVSNRAKNISGQSPARTSSDPGTNTTTEDHKIMASENSSAMVQVHSQGREAAVSHLTTLATISTSPQPPTTKPGPDNSTHNTPVYKLDISEATQVEQHHRRTDNDSTASDTPPATTAAGPLKAENTNTSKGTDLLDPATTTSPQNHSETAGNNNTHHQDTGEESASSGKLGLITNTIAGVAGLITGGRRARREAIVNAQPKCNPNLHYWTTQDEGAAIGLAWIPYFGPAAEGIYIEGLMHNQDGLICGLRQLANETTQALQLFLRATTELRTFSILNRKAIDFLLQRWGGTCHILGPDCCIEPHDWTKNITDKIDQIIHDFVDKTLPDQGDNDNWWTGWRQWIPAGIGVTGVIIAVIALFCICKFVF

SEQ ID NO: 14 - protein, 676 aa, Ebola virus
MGGLSLLQLPRDKFRKSSFFVWVIILFQKAFSMPLGVVTNSTLEVTEIDQLVCKDHLASTDQLKSVGLNLEGSGVSTDIPSATKRWGFRSGVPPKVVSYEAGEWAENCYNLEIKKPDGSECLPPPPDGVRGFPRCRYVHKAQGTGPCPGDYAFHKDGAFFLYDRLASTVIYRGVNFAEGVIAFLILAKPKETFLQSPPIREAVNYTENTSSYYATSYLEYEIENFGAQHSTTLFKIDNNTFVRLDRPHTPQFLFQLNDTIHLHQQLSNTTGRLIWTLDANINADIGEWAFWENKKNLSEQLRGEELSFEALSLNETEDDDAASSRITKGRISDRATRKYSDLVPKNSPGMVPLHIPEGETTLPSQNSTEGRRVGVNTQETITETAATIIGTNGNHMQISTIGIRPSSSQIPSSSPTTAPSPEAQTPTTHTSGPSVMATEEPTTPPGSSPGPTTEAPTLTTPENITTAVKTVLPQESTSNGLITSTVTGILGSLGLRKRSRRQTNTKATGKCNPNLHYWTAQEQHNAAGIAWIPYFGPGAEGIYTEGLMHNQNALVCGLRQLANETTQALQLFLRATTELRTYTILNRKAIDFLLRRWGGTCRILGPDCCIEPHDWTKNITDKINQIIHDFIDNPLPNQDNDDNWWTGWRQWIPAGIGITGIIIAIIALLCVCKLLC

SEQ ID NO: 15 - protein, 676 aa, Ebola virus
MVTSGILQLPRERFRKTSFFVWVIILFHKVFPIPLGVVHNNTLQVSDIDKLVCRDKLSSTSQLKSVGLNLEGNGVATDVPTATKRWGFRAGVPPKVVNYEAGEWAENCYNLDIKKADGSECLPEAPEGVRGFPRCRYVHKVSGTGPCPEGFAFHKEGAFFLYDRLASTIIYRSTTFSEGVVAFLILPKTKKDFFQSPPLHEPANMTTDPSSYYHTVTLNYVADNFGTNMTNFLFQVDHLTYVQLEPRFTPQFLVQLNETIYTNGRRSNTTGTLIWKVNPTVDTGVGEWAFWENKKNFTKTLSSEELSVILVPRAQDPGSNQKTKVTPTSFANNQTSKNHEDLVPKDPASVVQVRDLQRENTVPTSPLNTVPTTLIPDTMEEQTTSHYELPNISGNHQERNNTAHPETLANNPPDNTTPSTPPQDGERTSSHTTPSPRPVPTSTIHPTTRETQIPTTMITSHDTDSNRPNPIDISESTEPGLLTNTIRGVANLLTGSRRTRREITLRTQAKCNPNLHYWTTQDEGAAIGLAWIPYFGPAAEGIYTEGIMHNQNGLICGLRQLANETTQALQLFLRATTELRTFSILNRKAIDFLLQRWGGTCHILGPDCCIEPHDWTKNITDKIDQIIHDFIDKPLPDQTDNDNWWTGWRQWVPAGIGITGVIIAVIALLCICKFLL

SEQ ID NO: 16 - protein, 676 aa, Ebola virus
MGASGILQLPRERFRKTSFFVWVIILFHKVFSIPLGVVHNNTLQVSDIDKFVCRDKLSSTSQLKSVGLNLEGNGVATDVPTATKRWGFRAGVPPKVVNCEAGEWAENCYNLAIKKVDGSECLPEAPEGVRDFPRCRYVHKVSGTGPCPGGLAFHKEGAFFLYDRLASTIIYRGTTFAEGVIAFLILPKARKDFFQSPPLHEPANMTTDPSSYYHTTTINYVVDNFGTNTTEFLFQVDHLTYVQLEARFTPQFLVLLNETIYSDNRRSNTTGKLIWKINPTVDTSMGEWAFWENKKNFTKTLSSEELSFVPVPETQNQVLDTTATVSPPISAHNHAAEDHKELVSEDSTPVVQMQNIKGKDTMPTTVTGVPTTTPSPFPINARNTDHTKSFIGLEGPQEDHSTTQPAKTTSQPTNSTESTTLNPTSEPSSRGTGPSSPTVPNTTESHAELGKTTPTTLPEQHTAASAIPRAVHPDELSGPGFLTNTIRGVTNLLTGSRRKRRDVTPNTQPKCNPNLHYWTALDEGAAIGLAWIPYFGPAAEGIYTEGIMENQNGLICGLRQLANETTQALQLFLRATTELRTFSILNRKAIDFLLQRWGGTCHILGPDCCIEPQDWTKNITDKIDQIIHDFVDNNLPNQNDGSNWWTGWKQWVPAGIGITGVIIAIIALLCICKFML

SEQ ID NO: 17 - protein, 677 aa, Ebola virus
MGSGYQLLQLPRERFRKTSFLVWAIILFQRAISMPLGIVTNSTLKATEIDQLVCRDKLSSTSQLKSVGLNLEGNGIATDVPSATKRWGFRSGVPPKVVSYEAGEWAENCYNLEIKKSDGSECLPPPPDGVRGFPRCRYVHKVQGTGPCPGDLAFHKNGAFFLYDRLASTVIYRGTTFAEGVIAFLILSEPRKHFWKATPAHEPVNTTDDSTSYYITLTLSYEMSNFGGEESNTLFKVDNHTYVQLDRPHTPQFLVQLNETLRRNNRLSNSTGRLTWTLDPKIEPNVGEWAFWETKKNFSKQLQGENLHFQILSTHTNNSSDQSPAGTVQGKISYHPPTNNSELVPTDSPPVVSVLTAGRTEEMSTQGLTNGETITGFTANPMTTTIALSPTMTSKVDNNVPSEQPNNTTSIEDSPPSASNETIDHSEMNSIQGSNNSTQSPQTKTKPAPTASLMTLGPQETANSSKPGTSPGSAAEPSQPGLTINTVSKVADSLSPTRKQKRSVRQNTANECNPDLHYWTAVDEGAAVGLAWIPYFGPAAEGIYIEGVMHNQNGLICGLRQLANETTQALQLFLRATTELRTYSLLNRKAIDFLLQRWGGTCRILGPSCCIEPHDWTKNITDEINQIKHDFIDNPLPDHGDDLNLWTGWRQWIPAGIGIIGVIIAITALLCICKILC

SEQ ID NO: 18 - protein, 681 aa, Marburg virus
MKTIYFLISLILIQSIKTLPVLEIASNSQPQDVDSVCSGTLQKTEDVHLMGFTLSGQKVADSPLEASKRWAFRTGVPPKNVEYTEGEEAKTCYNISVTDPSGKSLLLDPPSNIRDYPKCKTVHHIQGQNPHAQGIALHLWGAFFLYDRVASTTMYRGKVFTEGNIAAMIVNKTVHRMIFSRQGQGYRHMNLTSTNKYWTSSNETQRNDTGCFGILQEYNSTNNQTCPPSLKPPSLPTVTPSIHSTNTQINTAKSGTMNPSSDDEDLMISGSGSGEQGPHTTLNVVTEQKQSSTILSTPSLHPSTSQHEQNSTNPSRHAVTEHNGTDPTTQPATLLNNTNTTPTYNTLKYNLSTPSPPTRNITNNDTQRELAESEQTNAQLNTTLDPTENPTTGQDTNSTTNIIMTTSDITSKHPTNSSPDSSPTTRPPIYFRKKRSIFWKEGDIFPFLDGLINTEIDFDPIPNTETIFDESPSFNTSTNEEQHTPPNISLTFSYFPDKNGDTAYSGENENDCDAELRIWSVQEDDLAAGLSWIPFFGPGIEGLYTAGLIKNQNNLVCRLRRLANQTAKSLELLLRVTTEERTFSLINRHAIDFLLTRWGGTCKVLGPDCCIGIEDLSKNISEQIDKIRKDEQKEETGWGLGGKWWTSDWGVLTNLGILLLLSIAVLIALSCICRIFTKYIG

SEQ ID NO: 19 - protein, 681 aa, Marburg virus
MKTTCLLISLILIQGVKTLPILEIASNIQPQNVDSVCSGTLQKTEDVHLMGFTLSGQKVADSPLEASKRWAFRAGVPPKNVEYTEGEEAKTCYNISVTDPSGKSLLLDPPTNIRDYPKCKTIHHIQGQNPHAQGIALHLWGAFFLYDRIASTTMYRGKVFTEGNIAAMIVNKTVHKMIFSRQGQGYRHMNLTSTNKYWTSSNGTQTNDTGCFGTLQEYNSTKNQTCAPSKKPLPLPTAHPEVKLTSTSTDATKLNTTDPNSDDEDLTTSGSGSGEQEPYTTSDAATKQGLSSTMPPTPSPQPSTPQQGGNNTNHSQGVVTEPGKTNTTAQPSMPPHNTTTISTNNTSKHNLSTPSVPIQNATNYNTQSTAPENEQTSAPSKTTLLPTENPTTAKSTNSTKSPTTTVPNTTNKYSTSPSPTPDSTAQHLVYFRRKRNILWREGDMFPFLDGLINAPIDFDPVPNTKTIFDESSSSGASAEEDQHASPNISLTLSYFPKVNENTAHSGENENDCDAELRIWSVQEDDLAAGLSWIPFFGPGIEGLYTAGLIKNQNNLVCRLRRLANQTAKSLELLLRVTTEERTFSLINRHAIDFLLARWGGTCKVLGPDCCIGIEDLSRNISEQIDQIKKDEQKEGTGWGLGGKWWTSDWGVLTNLGILLLLSIAVLIALSCICRIFTKYIG

SEQ ID NO: 20 - protein, 118 aa, rhesus macaque
EVQLVQSGGGLVQPGGSMRLSCEASGLSLSDYFMHWVRQAQGKGLEWIGLIQTKAFTYKTEYPAAVKGRFTISRDDSKNTLYLQMSSLKPEDTALYYCIAVTPDFYYWGQGVLVTVSS

SEQ ID NO: 21 - protein, 110 aa, rhesus macaque
DVVMTQSPSFLSASVGDRVTITCRASQDITINLNWFQHKPGKAPKRLIYVASRLERGVPSRFSGSGSGTEFTLTISSLQPEDFATYYCQQYNNYPLTFGPGTKLDIKRTV

SEQ ID NO: 22 - protein, 10 aa, rhesus macaque
GLSLSDYFMH

SEQ ID NO: 23 - protein, 10 aa, rhesus macaque
IQTKAFTYKT

SEQ ID NO: 24 - protein, 9 aa, rhesus macaque
IAVTPDFYY

SEQ ID NO: 25 - protein, 6 aa, rhesus macaque
QDITIN

SEQ ID NO: 26 - protein, 3 aa, rhesus macaque
VAS

SEQ ID NO: 27 - protein, 9 aa, rhesus macaque
QQYNNYPLT

SEQ ID NO: 28 - protein, 119 aa, cynomolgus macaque
QVQLQESGPGLVKPSETLSLTCAVSGGSISGGYYYWSWIRQPPGKGLEWIGNIYNSASTYYNPSLKSRVTISKDTSKNQFSLKLSSVTAADTAVYYCARGVVITGLDSWGQGVVVTVSS

SEQ ID NO: 29 - protein, 106 aa, cynomolgus macaque
DIQMTQSPSSLSASVGDRVTITCRASQGISSYLAWYQQKPGKAPKLLIYDASNLQSGVPSRFSGSGSGTDFTLTISSLQPEDFATYYCQQHNSYPLTFGGGTKVEI

SEQ ID NO: 30 - protein, 7 aa, Ebola virus
QLRSVGL

SEQ ID NO: 31 - protein, 7 aa, Ebola virus
PNLHYWT

SEQ ID NO: 32 - protein, 8 aa, Ebola virus
YTEGLMHN

SEQ ID NO: 33 - protein, 7 aa, Marburg virus
DVHLMGF

SEQ ID NO: 34 - protein, 7 aa, Marburg virus
AELRIWS

SEQ ID NO: 35 - protein, 8 aa, Marburg virus
YTAGLIKN